European Patent Application EP 4 495 132 A1, published January 22, 2025. Title: Target gene expression control system comprising dxCas9 and CRP derivative and preparation method therefor. Applicant: 한국화학연구원. The sequence listing filed with the application follows.

SEQUENCE LISTING (36 sequences)

SEQ ID NO: 1 - protein, 1368 aa, synthetic construct
MDKKYSIGLAIGTNSVGWAVITDEYKVPSKKFKVLGNTDRHSIKKNLIGALLFDSGETAEATRLKRTARRRYTRRKNRICYLQEIFSNEMAKVDDSFFHRLEESFLVEEDKKHERHPIFGNIVDEVAYHEKYPTIYHLRKKLVDSTDKADLRLIYLALAHMIKFRGHFLIEGDLNPDNSDVDKLFIQLVQTYNQLFEENPINASGVDAKAILSARLSKSRRLENLIAQLPGEKKNGLFGNLIALSLGLTPNFKSNFDLAEDTKLQLSKDTYDDDLDNLLAQIGDQYADLFLAAKNLSDAILLSDILRVNTEITKAPLSASMIKLYDEHHQDLTLLKALVRQQLPEKYKEIFFDQSKNGYAGYIDGGASQEEFYKFIKPILEKMDGTEELLVKLNREDLLRKQRTFDNGIIPHQIHLGELHAILRRQEDFYPFLKDNREKIEKILTFRIPYYVGPLARGNSRFAWMTRKSEETITPWNFEKVVDKGASAQSFIERMTNFDKNLPNEKVLPKHSLLYEYFTVYNELTKVKYVTEGMRKPAFLSGDQKKAIVDLLFKTNRKVTVKQLKEDYFKKIECFDSVEISGVEDRFNASLGTYHDLLKIIKDKDFLDNEENEDILEDIVLTLTLFEDREMIEERLKTYAHLFDDKVMKQLKRRRYTGWGRLSRKLINGIRDKQSGKTILDFLKSDGFANRNFIQLIHDDSLTFKEDIQKAQVSGQGDSLHEHIANLAGSPAIKKGILQTVKVVDELVKVMGRHKPENIVIEMARENQTTQKGQKNSRERMKRIEEGIKELGSQILKEHPVENTQLQNEKLYLYYLQNGRDMYVDQELDINRLSDYDVDAIVPQSFLKDDSIDNKVLTRSDKNRGKSDNVPSEEVVKKMKNYWRQLLNAKLITQRKFDNLTKAERGGLSELDKAGFIKRQLVETRQITKHVAQILDSRMNTKYDENDKLIREVKVITLKSKLVSDFRKDFQFYKVREINNYHHAHDAYLNAVVGTALIKKYPKLESEFVYGDYKVYDVRKMIAKSEQEIGKATAKYFFYSNIMNFFKTEITLANGEIRKRPLIETNGETGEIVWDKGRDFATVRKVLSMPQVNIVKKTEVQTGGFSKESILPKRNSDKLIARKKDWDPKKYGGFDSPTVAYSVLVVAKVEKGKSKKLKSVKELLGITIMERSSFEKNPIDFLEAKGYKEVKKDLIIKLPKYSLFELENGRKRMLASAGVLQKGNELALPSKYVNFLYLASHYEKLKGSPEDNEQKQLFVEQHKHYLDEIIEQISEFSKRVILADANLDKVLSAYNKHRDKPIREQAENIIHLFTLTNLGAPAAFKYFDTTIDRKRYTSTKEVLDATLIHQSITGLYETRIDLSQLGGD

SEQ ID NO: 2 - protein, 10 aa, synthetic construct
GGGAGGGGAG

SEQ ID NO: 3 - DNA, 65 bp, synthetic construct
  source 1..65: mol_type = other DNA
agcaggatcaccataagaattcaaaagatctaaagaggagaaaggatctatggacaagaagtact

SEQ ID NO: 4 - DNA, 46 bp, synthetic construct
  source 1..46: mol_type = other DNA
ctagactagtgccggcgccgccgccgtctccaccgagctgagagag

SEQ ID NO: 5 - protein, 210 aa, Escherichia coli
MVLGKPQTDPTLEWFLSHCHIHKYPSKSTLIHQGEKAETLYYIVKGSVAVLIKDEEGKEMILSYLNQGDFIGELGLFEEGQERSAWVRAKTACEVAEISYKKFRQLIQVNPDILMRLSAQMARRLQVTSEKVGNLAFLDVTGRIAQTLLNLAKQPDAMTHPDGMQIKITRQEIGQIVGCSRETVGRILKMLEDQNLISAHGKTIVVYGTR

SEQ ID NO: 6 - protein, 180 aa, synthetic construct
MVLGKPQTDPTLEWFLSHCHIHKYPSKSTLIHQGEKAETLYYIVKGSVAVLIKDEEGKEMILSYLNQGDFIGELGLFEEGQERSAWVRAKTACEVAEISYKKFRQLIQVNPDILMRLSAQMARRLQVTSEKVGNLAFLDVTGRIAQTLLNLAKQPDAMTHPDGMQIKITRQEIGQIVGCS

SEQ ID NO: 7 - protein, 139 aa, synthetic construct
MVLGKPQTDPTLEWFLSHCHIHKYPSKSTLIHQGEKAETLYYIVKGSVAVLIKDEEGKEMILSYLNQGDFIGELGLFEEGQERSAWVRAKTACEVAEISYKKFRQLIQVNPDILMRLSAQMARRLQVTSEKVGNLAFLD

SEQ ID NO: 8 - protein, 45 aa, synthetic construct
AFLDVTGRIAQTLLNLAKQPDAMTHPDGMQIKITRQEIGQIVGCS

SEQ ID NO: 9 - protein, 60 aa, synthetic construct
STLIHQGEKAETLYYIVKGSVAVLIKDEEGKEMILSYLNQGDFIGELGLFEEGQERSAWV

SEQ ID NO: 10 - DNA, 34 bp, synthetic construct
  source 1..34: mol_type = other DNA
cggcggcggcgccggcatggtgcttggcaaaccg

SEQ ID NO: 11 - DNA, 35 bp, synthetic construct
  source 1..35: mol_type = other DNA
cggcggcggcgccggcgcgttcctcgacgtgacgg

SEQ ID NO: 12 - DNA, 36 bp, synthetic construct
  source 1..36: mol_type = other DNA
cggcggcggcgccggcagcacgcttattcaccaggg

SEQ ID NO: 13 - DNA, 56 bp, synthetic construct
  source 1..56: mol_type = other DNA
gaggactagtgccggttagtggtggtggtggtggtgacgagtgccgtaaacgacga

SEQ ID NO: 14 - DNA, 58 bp, synthetic construct
  source 1..58: mol_type = other DNA
gaggactagtgccggttagtggtggtggtggtggtgagaacagccgacaatctgacca

SEQ ID NO: 15 - DNA, 55 bp, synthetic construct
  source 1..55: mol_type = other DNA
gaggactagtgccggttagtggtggtggtggtggtggtcgaggaacgccaggttg

SEQ ID NO: 16 - DNA, 55 bp, synthetic construct
  source 1..55: mol_type = other DNA
gaggactagtgccggttagtggtggtggtggtggtgggcggttttcgcacgtacc

SEQ ID NO: 17 - DNA, 35 bp, synthetic construct
  source 1..35: mol_type = other DNA
aaggagatatacatatggcctacggtatccaccgg

SEQ ID NO: 18 - DNA, 42 bp, synthetic construct
  source 1..42: mol_type = other DNA
tcttctcctttactcatatgacctttctcctctttaatgaat

SEQ ID NO: 19 - DNA, 35 bp, synthetic construct; identical to SEQ ID NO: 17
  source 1..35: mol_type = other DNA

SEQ ID NO: 20 - DNA, 83 bp, synthetic construct
  source 1..83: mol_type = other DNA
tcttctcctttactcatatgacctttctcctctttaatgaattcgctagcacaatccctaggactgagctagctgtcaagtcc

SEQ ID NO: 21 - DNA, 102 bp, synthetic construct
  source 1..102: mol_type = other DNA
gggaaatgtgggatcgccggcttgacagctagctcagtcctaggtataatgctagcgaattcattaaagaggagaaaggtaccatggtaagtaagggtgaag

SEQ ID NO: 22 - DNA, 98 bp, synthetic construct
  source 1..98: mol_type = other DNA
tggcgatatcggatccaaaaaacccctcaagacccgtttagaggccccaaggggttatgctagcccgggagatctttatttgtacaattcgtccattc

SEQ ID NO: 23 - RNA, 20 nt, synthetic construct
  source 1..20: mol_type = other RNA
ccggagacctatggcagcct

SEQ ID NO: 24 - RNA, 20 nt, synthetic construct
  source 1..20: mol_type = other RNA
catctaattcaacaagaatt

SEQ ID NO: 25 - RNA, 20 nt, synthetic construct
  source 1..20: mol_type = other RNA
ttcttcacccttacttacca

SEQ ID NO: 26 - DNA, 39 bp, synthetic construct
  source 1..39: mol_type = other DNA
actaaccggcactagctcgagtaaggatctccaggcatc

SEQ ID NO: 27 - DNA, 55 bp, synthetic construct
  source 1..55: mol_type = other DNA
aggctgccataggtctccggactagtattatacctaggactgagctagctgtcaa

SEQ ID NO: 28 - DNA, 55 bp, synthetic construct
  source 1..55: mol_type = other DNA
taatactagtccggagacctatggcagcctgttttagagctagaaatagcaagtt

SEQ ID NO: 29 - DNA, 55 bp, synthetic construct
  source 1..55: mol_type = other DNA
aattcttgttgaattagatgactagtattatacctaggactgagctagctgtcaa

SEQ ID NO: 30 - DNA, 55 bp, synthetic construct
  source 1..55: mol_type = other DNA
taatactagtcatctaattcaacaagaattgttttagagctagaaatagcaagtt

SEQ ID NO: 31 - DNA, 55 bp, synthetic construct
  source 1..55: mol_type = other DNA
tggtaagtaagggtgaagaagctagcattatacctaggactgagctagctgtcaa

SEQ ID NO: 32 - DNA, 55 bp, synthetic construct
  source 1..55: mol_type = other DNA
taatgctagcttcttcacccttacttaccagttttagagctagaaatagcaagtt

SEQ ID NO: 33 - DNA, 43 bp, synthetic construct
  source 1..43: mol_type = other DNA
ttcctcgaggcggccgcaaaaaagcaccgactcggtgccactt

SEQ ID NO: 34 - DNA, 10023 bp, synthetic construct
  source 1..10023: mol_type = other DNA
ggcgcccaatacgcaaaccgcctctccccgcgcgttggccgattcattaatgcagctggcacgacaggtttcccgactggaaagcgggcagtgagcgcaacgcaattaatgtaagttagctcactcattaggcaccgggatctcgaccgatgcccttgagagccttcaacccagtcagctccttccggtgggcgcggggcatgactaacatgagaattacaacttatatcgtatggggctgacttcaggtgctacatttgaagagataaattgcactgaaatctagaaatattttatctgattaataagatgatcttcttgagatcgttttggtctgcgcgtaatctcttgctctgaaaacgaaaaaaccgccttgcagggcggtttttcgaaggttctctgagctaccaactctttgaaccgaggtaactggcttggaggagcgcagtcaccaaaacttgtcctttcagtttagccttaaccggcgcatgacttcaagactaactcctctaaatcaattaccagtggctgctgccagtggtgcttttgcatgtctttccgggttggactcaagacgatagttaccggataaggcgcagcggtcggactgaacggggggttcgtgcatacagtccagcttggagcgaactgcctacccggaactgagtgtcaggcgtggaatgagacaaacgcggccataacagcggaatgacaccggtaaaccgaaaggcaggaacaggagagcgcacgagggagccgccaggggaaacgcctggtatctttatagtcctgtcgggtttcgccaccactgatttgagcgtcagatttcgtgatgcttgtcaggggggcggagcctatggaaaaacggctttgccgcggccctctcacttccctgttaagtatcttcctggcatcttccaggaaatctccgccccgttcgtaagccatttccgctcgccgcagtcgaacgaccgagcgtagcgagtcagtgagcgaggaagcggaatatatcctgtatcacatattctgctgacgcaccggtgcagccttttttctcctgccacatgaagcacttcactgacaccctcatcagtgccaacatagtaagccagtatacactccgctagcgctgatgtccggcggtgcttttgccgttacgcaccaccccgtcagtagctgaacaggagggacagctgatagaaacagaagccactggagcacctcaaaaacaccatcatacactaaatcagtaagttggcagcatcacccgacgcactttgcgccgaataaatacctgtgacggaagatcacttcgcagaataaataaatcctggtgtccctgttgataccgggaagccctgggccaacttttggcgaaaatgagacgttgatcggcacgtaagaggttccaactttcaccataatgaaataagatcactaccgggcgtattttttgagttatcgagattttcaggagctaaggaagctaaaatggagaaaaaaatcactggatataccaccgttgatatatcccaatggcatcgtaaagaacattttgaggcatttcagtcagttgctcaatgtacctataaccagaccgttcagctggatattacggcctttttaaagaccgtaaagaaaaataagcacaagttttatccggcctttattcacattcttgcccgcctgatgaatgctcatccggagttccgtatggcaatgaaagacggtgagctggtgatatgggatagtgttcacccttgttacaccgttttccatgagcaaactgaaacgttttcatcgctctggagtgaataccacgacgatttccggcagtttctacacatatattcgcaagatgtggcgtgttacggtgaaaacctggcctatttccctaaagggtttattgagaatatgtttttcgtctcagccaatccctgggtgagtttcaccagttttgatttaaacgtggccaatatggacaacttcttcgcccccgttttcactatgggcaaatattatacgcaaggcgacaaggtgctgatgccgctggcgattcaggttcatcatgccgtctgtgatggcttccatgtcggcagaatgcttaatgaattacaacagtactgcgatgagtggcagggcggggcgtaatttttttaaggcagttattggtgcccttaaacgcctggtgctacgcctgaataagtgataataagcggatgaatggcagaaattcgaaagcaaattcgacccggtcgtcggttcagggcagggtcgttaaatagccgcttatgtctattgctggtttaccggtttattgactaccggaagcagtgtgaccgtgtgcttctcaaatgcctgaggtttcagcaaaaaacccctcaagacccgtttagaggccccaaggggttatgctagttattgctcagcggtggcagcagcctaggttaattaagctgcgctagtagacgagtccatgtgctggcgttcaaatttcgcagcagcggtttctttaccagactcgaggcgaattaatctttctgcgaattgagatgacgccactggctgggcgtcatcccggtttcccgggtaaacaccaccgaaaaatagttactatcttcaaagccacattcggtcgaaatatcactgattaacaggcggctatgctggagaagatattgcgcatgacacactctgacctgtcgcagatattgattgatggtcattccagtctgctggcgaaattgctgacgcaaaacgcgctcactgcacgatgcctcatcacaaaatttatccagcgcaaagggacttttcaggctagccgccagccgggtaatcagcttatccagcaacgtttcgctggatgttggcggcaacgaatcactggtgtaacgatggcgattcagcaacatcaccaactgcccgaacagcaactcagccatttcgttagcaaacggcacatgctgactactttcatgctcaagctgaccgataacctgccgcgcctgcgccatccccatgctacctaagcgccagtgtggttgccctgcgctggcgttaaatcccggaatcgccccctgccagtcaagattcagcttcagacgctccgggcaataaataatattctgcaaaaccagatcgttaacggaagcgtaggagtgtttatcgtcagcatgaatgtaaaagagatcgccacgggtaatgcgataagggcgatcgttgagtacatgcaggccattaccgcgccagacaatcaccagctcacaaaaatcatgtgtatgttcagcaaagacatcttgcggataacggtcagccacagcgactgcctgctggtcgctggcaaaaaaatcatctttgagaagttttaactgatgcgccaccgtggctacctcggccagagaacgaagttgattattcgcaatatggcgtacaaatacgttgagaagattcgcgttattgcagaaagccatcccgtccctggcgaatatcacgcggtgaccagttaaactctcggcgaaaaagcgtcgaaaagtggttactgtcgctgaatccacagcgataggcgatgtcagtaacgctggcctcgctgtggcgtagcagatgtcgggctttcatcagtcgcaggcggttcaggtatcgctgaggcgtcagtcccgtttgctgcttaagctgccgatgtagcgtacgcagtgaaagagaaaattgatccgccacggcatcccaattcacctcatcggcaaaatggtcctccagccaggccagaagcaagttgagacgtgatgcgctgttttccaggttctcctgcaaactgcttttacgcagcaagagcagtaattgcataaacaagatctcgcgactggcggtcgagggtaaatcattttccccttcctgctgttccatctgtgcaaccagctgtcgcacctgctgcaatacgctgtggttaacgcgccagtgagacggatactgcccatccagctcttgtggcagcaactgattcagcccggcgagaaactgaaatcgatccggcgagcgatacagcacattggtcagacacagattatcggtatgttcatacagatgccgatcatgatcgcgtacgaaacagaccgtgccaccggtgatggtatagggctgcccattaaacacatgaatacccgtgccatgttcgacaatcacaatttcatgaaaatcatgatgatgttcaggaaaatccgcctgcgggagccggggttctatcgccacggacgcgttaccagacggaaaaaaatccacactatgtaatacggtcatactggcctcctgatgtcgtcaacacggcgaaatagtaatcacgaggtcaggttcttaccttaaattttcgacggaaaaccacgtaaaaaacgtcgatttttcaagatacagcgtgaattttcaggaaatgcggtgagcatcacatcaccacaattcagcaaattgtgaacatcatcacgttcatctttccctggttgccaatggcccattttcctgtcagtaacgagaaggtcgcgaattcaggcgctttttagactggtcgtaatgaaattcagcaggatcaccataagaattcaaaagatctaaagaggagaaaggatctatggacaagaagtactccattgggctcgctatcggcacaaacagcgtcggctgggccgtcattacggacgagtacaaggtgccgagcaaaaaattcaaagttctgggcaataccgatcgccacagcataaagaagaacctcattggcgccctcctgttcgactccggggagacggccgaagccacgcggctcaaaagaacagcacggcgcagatatacccgcagaaagaatcggatctgctacctgcaggagatctttagtaatgagatggctaaggtggatgactctttcttccataggctggaggagtcctttttggtggaggaggataaaaagcacgagcgccacccaatctttggcaatatcgtggacgaggtggcgtaccatgaaaagtacccaaccatatatcatctgaggaagaagcttgtagacagtactgataaggctgacttgcggttgatctatctcgcgctggcgcatatgatcaaatttcggggacacttcctcatcgagggggacctgaacccagacaacagcgatgtcgacaaactctttatccaactggttcagacttacaatcagcttttcgaagagaacccgatcaacgcatccggagttgacgccaaagcaatcctgagcgctaggctgtccaaatcccggcggctcgaaaacctcatcgcacagctccctggggagaagaagaacggcctgtttggtaatcttatcgccctgtccctcgggctgacccccaactttaaatctaacttcgacctggccgaagataccaagcttcaactgagcaaagacacctacgatgatgatctcgacaatctgctggcccagatcggcgaccagtacgcagacctttttttggcggcaaagaacctgtcagacgccattctgctgagtgatattctgcgagtgaacacggagatcaccaaagctccgctgagcgctagtatgatcaagctctatgatgagcaccaccaagacttgactttgctgaaggcccttgtcagacagcaactgcctgagaagtacaaggaaattttcttcgatcagtctaaaaatggctacgccggatacattgacggcggagcaagccaggaggaattttacaaatttattaagcccatcttggaaaaaatggacggcaccgaggagctgctggtaaagcttaacagagaagatctgttgcgcaaacagcgcactttcgacaatggaatcatcccccaccagattcacctgggcgaactgcacgctatcctcaggcggcaagaggatttctacccctttttgaaagataacagggaaaagattgagaaaatcctcacatttcggataccctactatgtaggccccctcgcccggggaaattccagattcgcgtggatgactcgcaaatcagaagagaccatcactccctggaacttcgagaaagtcgtggataagggggcctctgcccagtccttcatcgaaaggatgactaactttgataaaaatctgcctaacgaaaaggtgcttcctaaacactctctgctgtacgagtacttcacagtttataacgagctcaccaaggtcaaatacgtcacagaagggatgagaaagccagcattcctgtctggagatcagaagaaagctattgtggacctcctcttcaagacgaaccggaaagttaccgtgaaacagctcaaagaagactatttcaaaaagattgaatgtttcgactctgttgaaatcagcggagtggaggatcgcttcaacgcatccctgggaacgtatcacgatctcctgaaaatcattaaagacaaggacttcctggacaatgaggagaacgaggacattcttgaggacattgtcctcacccttacgttgtttgaagatagggagatgattgaagaacgcttgaaaacttacgctcatctcttcgacgacaaagtcatgaagcagctcaagaggcgccgatatacaggatgggggcggctgtcaagaaaactgatcaatgggatccgagacaagcagagtggaaagacaatcctggattttcttaagtccgatggatttgccaaccggaacttcattcagttgatccatgatgactctctcacctttaaggaggacatccagaaagcacaagtttctggccagggggacagtcttcacgagcacatcgctaatcttgcaggtagcccagctatcaaaaagggaatactgcagaccgttaaggtcgtggatgaactcgtcaaagtaatgggaaggcataagcccgagaatatcgttatcgagatggcccgagagaaccaaaccacccagaagggacagaagaacagtagggaaaggatgaagaggattgaagagggtataaaagaactggggtcccaaatccttaaggaacacccagttgaaaacacccagcttcagaatgagaagctctacctgtactacctgcagaacggcagggacatgtacgtggatcaggaactggacatcaatcggctctccgactacgacgtggacgctatcgtgccccagtcttttctcaaagatgattctattgataataaagtgttgacaagatccgataaaaacagagggaagagtgataacgtcccctcagaagaagttgtcaagaaaatgaaaaattattggcggcagctgctgaacgccaaactgatcacacaacggaagttcgataatctgactaaggctgaacgaggtggcctgtctgagttggataaagccggtttcatcaaaaggcagcttgttgagacacgccagatcaccaagcacgtggcccaaattctcgattcacgcatgaacaccaagtacgatgaaaatgacaaactgattcgagaggtgaaagttattactctgaagtctaagctggtctcagatttcagaaaggactttcagttttataaggtgagagagatcaacaattaccaccatgcgcatgatgcctacctgaatgcagtggtaggcactgcacttatcaaaaaatatcccaagcttgaatctgaatttgtttacggagactataaagtgtacgatgttaggaaaatgatcgcaaagtctgagcaggaaataggcaaggccaccgctaagtacttcttttacagcaatattatgaattttttcaagaccgagattacactggccaatggagagattcggaagcgaccacttatcgaaacaaacggagaaacaggagaaatcgtgtgggacaagggtagggatttcgcgacagtccggaaggtcctgtccatgccgcaggtgaacatcgttaaaaagaccgaagtacagaccggaggtttctccaaggaaagtatcctcccgaaaaggaacagcgacaagctgatcgcacgcaaaaaagattgggaccccaagaaatacggcggattcgattctcctacagtcgcttacagtgtactggttgtggccaaagtggagaaagggaagtctaaaaaactcaaaagcgtcaaggaactgctgggcatcacaatcatggagcgatcaagcttcgaaaaaaaccccatcgactttctcgaggcgaaaggatataaagaggtcaaaaaagacctcatcattaagcttcccaagtactctctctttgagcttgaaaacggccggaaacgaatgctcgctagtgcgggcgtgctgcagaaaggtaacgagctggcactgccctctaaatacgttaatttcttgtatctggccagccactatgaaaagctcaaagggtctcccgaagataatgagcagaagcagctgttcgtggaacaacacaaacactaccttgatgagatcatcgagcaaataagcgaattctccaaaagagtgatcctcgccgacgctaacctcgataaggtgctttctgcttacaataagcacagggataagcccatcagggagcaggcagaaaacattatccacttgtttactctgaccaacttgggcgcgcctgcagccttcaagtacttcgacactaccatagacagaaagcggtacacctctacaaaggaggtcctggacgccacactgattcatcagtcaattacggggctctatgaaacaagaatcgacctctctcagctcggtggagacggcggcggcgccggcggcggcggcgccggcatggtgcttggcaaaccgcaaacagacccgactctcgaatggttcttgtctcattgccacattcataagtacccatccaagagcacgcttattcaccagggtgaaaaagcggaaacgctgtactacatcgttaaaggctctgtggcagtgctgatcaaagacgaagagggtaaagaaatgatcctctcctatctgaatcagggtgattttattggcgaactgggcctgtttgaagagggccaggaacgtagcgcatgggtacgtgcgaaaaccgcctgtgaagtggctgaaatttcgtacaaaaaatttcgccaattgattcaggtaaacccggacattctgatgcgtttgtctgcacagatggcgcgtcgtctgcaagtcacttcagagaaagtgggcaacctggcgttcctcgacgtgacgggccgcattgcacagactctgctgaatctggcaaaacaaccagacgctatgactcacccggacggtatgcaaatcaaaattacccgtcaggaaattggtcagattgtcggctgttctcaccaccaccaccaccactaaccggcactagctcgagtaaggatctccaggcatcaaataaaacgaaaggctcagtcgaaagactgggcctttcgttttatctgttgtttgtcggtgaacgctctctactagagtcacactggctcaccttcgggtgggcctttctgcgtttatacctagggatatattccgcttcctcggcgaccggttaaagatctttgacagctagctcagtcctaggtataatactagtccggagacctatggcagcctgttttagagctagaaatagcaagttaaaataaggctagtccgttatcaacttgaaaaagtggcaccgagtcggtgcttttttgcggccgcctcgaggaagcttgggcccgaacaaaaactcatctcagaagaggatctgaatagcgccgtcgaccatcatcatcatcatcattgagtttaaacggtctccagcttggctgttttggcggatgagagaagattttcagcctgatacagattaaatcagaacgcagaagcggtctgataaaacagaatttgcctggcggcagtagcgcggtggtcccacctgaccccatgccgaactcagaagtgaaacgccgtagcgccgatggtagtgtggggtctccccatgcgagagtagggaactgccaggcatcaaataaaacgaaaggctcagtcgaaagactgggcctttcgttttatctgttgtttgtcggtgaact

SEQ ID NO: 35 - DNA, 9973 bp, synthetic construct
  source 1..9973: mol_type = other DNA
ggcgcccaatacgcaaaccgcctctccccgcgcgttggccgattcattaatgcagctggcacgacaggtttcccgactggaaagcgggcagtgagcgcaacgcaattaatgtaagttagctcactcattaggcaccgggatctcgaccgatgcccttgagagccttcaacccagtcagctccttccggtgggcgcggggcatgactaacatgagaattacaacttatatcgtatggggctgacttcaggtgctacatttgaagagataaattgcactgaaatctagaaatattttatctgattaataagatgatcttcttgagatcgttttggtctgcgcgtaatctcttgctctgaaaacgaaaaaaccgccttgcagggcggtttttcgaaggttctctgagctaccaactctttgaaccgaggtaactggcttggaggagcgcagtcaccaaaacttgtcctttcagtttagccttaaccggcgcatgacttcaagactaactcctctaaatcaattaccagtggctgctgccagtggtgcttttgcatgtctttccgggttggactcaagacgatagttaccggataaggcgcagcggtcggactgaacggggggttcgtgcatacagtccagcttggagcgaactgcctacccggaactgagtgtcaggcgtggaatgagacaaacgcggccataacagcggaatgacaccggtaaaccgaaaggcaggaacaggagagcgcacgagggagccgccaggggaaacgcctggtatctttatagtcctgtcgggtttcgccaccactgatttgagcgtcagatttcgtgatgcttgtcaggggggcggagcctatggaaaaacggctttgccgcggccctctcacttccctgttaagtatcttcctggcatcttccaggaaatctccgccccgttcgtaagccatttccgctcgccgcagtcgaacgaccgagcgtagcgagtcagtgagcgaggaagcggaatatatcctgtatcacatattctgctgacgcaccggtgcagccttttttctcctgccacatgaagcacttcactgacaccctcatcagtgccaacatagtaagccagtatacactccgctagcgctgatgtccggcggtgcttttgccgttacgcaccaccccgtcagtagctgaacaggagggacagctgatagaaacagaagccactggagcacctcaaaaacaccatcatacactaaatcagtaagttggcagcatcacccgacgcactttgcgccgaataaatacctgtgacggaagatcacttcgcagaataaataaatcctggtgtccctgttgataccgggaagccctgggccaacttttggcgaaaatgagacgttgatcggcacgtaagaggttccaactttcaccataatgaaataagatcactaccgggcgtattttttgagttatcgagattttcaggagctaaggaagctaaaatggagaaaaaaatcactggatataccaccgttgatatatcccaatggcatcgtaaagaacattttgaggcatttcagtcagttgctcaatgtacctataaccagaccgttcagctggatattacggcctttttaaagaccgtaaagaaaaataagcacaagttttatccggcctttattcacattcttgcccgcctgatgaatgctcatccggagttccgtatggcaatgaaagacggtgagctggtgatatgggatagtgttcacccttgttacaccgttttccatgagcaaactgaaacgttttcatcgctctggagtgaataccacgacgatttccggcagtttctacacatatattcgcaagatgtggcgtgttacggtgaaaacctggcctatttccctaaagggtttattgagaatatgtttttcgtctcagccaatccctgggtgagtttcaccagttttgatttaaacgtggccaatatggacaacttcttcgcccccgttttcactatgggcaaatattatacgcaaggcgacaaggtgctgatgccgctggcgattcaggttcatcatgccgtctgtgatggcttccatgtcggcagaatgcttaatgaattacaacagtactgcgatgagtggcagggcggggcgtaatttttttaaggcagttattggtgcccttaaacgcctggtgctacgcctgaataagtgataataagcggatgaatggcagaaattcgaaagcaaattcgacccggtcgtcggttcagggcagggtcgttaaatagccgcttatgtctattgctggtttaccggtttattgactaccggaagcagtgtgaccgtgtgcttctcaaatgcctgaggtttcagcaaaaaacccctcaagacccgtttagaggccccaaggggttatgctagttattgctcagcggtggcagcagcctaggttaattaagctgcgctagtagacgagtccatgtgctggcgttcaaatttcgcagcagcggtttctttaccagactcgaggcgaattaatctttctgcgaattgagatgacgccactggctgggcgtcatcccggtttcccgggtaaacaccaccgaaaaatagttactatcttcaaagccacattcggtcgaaatatcactgattaacaggcggctatgctggagaagatattgcgcatgacacactctgacctgtcgcagatattgattgatggtcattccagtctgctggcgaaattgctgacgcaaaacgcgctcactgcacgatgcctcatcacaaaatttatccagcgcaaagggacttttcaggctagccgccagccgggtaatcagcttatccagcaacgtttcgctggatgttggcggcaacgaatcactggtgtaacgatggcgattcagcaacatcaccaactgcccgaacagcaactcagccatttcgttagcaaacggcacatgctgactactttcatgctcaagctgaccgataacctgccgcgcctgcgccatccccatgctacctaagcgccagtgtggttgccctgcgctggcgttaaatcccggaatcgccccctgccagtcaagattcagcttcagacgctccgggcaataaataatattctgcaaaaccagatcgttaacggaagcgtaggagtgtttatcgtcagcatgaatgtaaaagagatcgccacgggtaatgcgataagggcgatcgttgagtacatgcaggccattaccgcgccagacaatcaccagctcacaaaaatcatgtgtatgttcagcaaagacatcttgcggataacggtcagccacagcgactgcctgctggtcgctggcaaaaaaatcatctttgagaagttttaactgatgcgccaccgtggctacctcggccagagaacgaagttgattattcgcaatatggcgtacaaatacgttgagaagattcgcgttattgcagaaagccatcccgtccctggcgaatatcacgcggtgaccagttaaactctcggcgaaaaagcgtcgaaaagtggttactgtcgctgaatccacagcgataggcgatgtcagtaacgctggcctcgctgtggcgtagcagatgtcgggctttcatcagtcgcaggcggttcaggtatcgctgaggcgtcagtcccgtttgctgcttaagctgccgatgtagcgtacgcagtgaaagagaaaattgatccgccacggcatcccaattcacctcatcggcaaaatggtcctccagccaggccagaagcaagttgagacgtgatgcgctgttttccaggttctcctgcaaactgcttttacgcagcaagagcagtaattgcataaacaagatctcgcgactggcggtcgagggtaaatcattttccccttcctgctgttccatctgtgcaaccagctgtcgcacctgctgcaatacgctgtggttaacgcgccagtgagacggatactgcccatccagctcttgtggcagcaactgattcagcccggcgagaaactgaaatcgatccggcgagcgatacagcacattggtcagacacagattatcggtatgttcatacagatgccgatcatgatcgcgtacgaaacagaccgtgccaccggtgatggtatagggctgcccattaaacacatgaatacccgtgccatgttcgacaatcacaatttcatgaaaatcatgatgatgttcaggaaaatccgcctgcgggagccggggttctatcgccacggacgcgttaccagacggaaaaaaatccacactatgtaatacggtcatactggcctcctgatgtcgtcaacacggcgaaatagtaatcacgaggtcaggttcttaccttaaattttcgacggaaaaccacgtaaaaaacgtcgatttttcaagatacagcgtgaattttcaggaaatgcggtgagcatcacatcaccacaattcagcaaattgtgaacatcatcacgttcatctttccctggttgccaatggcccattttcctgtcagtaacgagaaggtcgcgaattcaggcgctttttagactggtcgtaatgaaattcagcaggatcaccatatggacaagaagtactccattgggctcgctatcggcacaaacagcgtcggctgggccgtcattacggacgagtacaaggtgccgagcaaaaaattcaaagttctgggcaataccgatcgccacagcataaagaagaacctcattggcgccctcctgttcgactccggggagacggccgaagccacgcggctcaaaagaacagcacggcgcagatatacccgcagaaagaatcggatctgctacctgcaggagatctttagtaatgagatggctaaggtggatgactctttcttccataggctggaggagtcctttttggtggaggaggataaaaagcacgagcgccacccaatctttggcaatatcgtggacgaggtggcgtaccatgaaaagtacccaaccatatatcatctgaggaagaagcttgtagacagtactgataaggctgacttgcggttgatctatctcgcgctggcgcatatgatcaaatttcggggacacttcctcatcgagggggacctgaacccagacaacagcgatgtcgacaaactctttatccaactggttcagacttacaatcagcttttcgaagagaacccgatcaacgcatccggagttgacgccaaagcaatcctgagcgctaggctgtccaaatcccggcggctcgaaaacctcatcgcacagctccctggggagaagaagaacggcctgtttggtaatcttatcgccctgtccctcgggctgacccccaactttaaatctaacttcgacctggccgaagataccaagcttcaactgagcaaagacacctacgatgatgatctcgacaatctgctggcccagatcggcgaccagtacgcagacctttttttggcggcaaagaacctgtcagacgccattctgctgagtgatattctgcgagtgaacacggagatcaccaaagctccgctgagcgctagtatgatcaagctctatgatgagcaccaccaagacttgactttgctgaaggcccttgtcagacagcaactgcctgagaagtacaaggaaattttcttcgatcagtctaaaaatggctacgccggatacattgacggcggagcaagccaggaggaattttacaaatttattaagcccatcttggaaaaaatggacggcaccgaggagctgctggtaaagcttaacagagaagatctgttgcgcaaacagcgcactttcgacaatggaatcatcccccaccagattcacctgggcgaactgcacgctatcctcaggcggcaagaggatttctacccctttttgaaagataacagggaaaagattgagaaaatcctcacatttcggataccctactatgtaggccccctcgcccggggaaattccagattcgcgtggatgactcgcaaatcagaagagaccatcactccctggaacttcgagaaagtcgtggataagggggcctctgcccagtccttcatcgaaaggatgactaactttgataaaaatctgcctaacgaaaaggtgcttcctaaacactctctgctgtacgagtacttcacagtttataacgagctcaccaaggtcaaatacgtcacagaagggatgagaaagccagcattcctgtctggagatcagaagaaagctattgtggacctcctcttcaagacgaaccggaaagttaccgtgaaacagctcaaagaagactatttcaaaaagattgaatgtttcgactctgttgaaatcagcggagtggaggatcgcttcaacgcatccctgggaacgtatcacgatctcctgaaaatcattaaagacaaggacttcctggacaatgaggagaacgaggacattcttgaggacattgtcctcacccttacgttgtttgaagatagggagatgattgaagaacgcttgaaaacttacgctcatctcttcgacgacaaagtcatgaagcagctcaagaggcgccgatatacaggatgggggcggctgtcaagaaaactgatcaatgggatccgagacaagcagagtggaaagacaatcctggattttcttaagtccgatggatttgccaaccggaacttcattcagttgatccatgatgactctctcacctttaaggaggacatccagaaagcacaagtttctggccagggggacagtcttcacgagcacatcgctaatcttgcaggtagcccagctatcaaaaagggaatactgcagaccgttaaggtcgtggatgaactcgtcaaagtaatgggaaggcataagcccgagaatatcgttatcgagatggcccgagagaaccaaaccacccagaagggacagaagaacagtagggaaaggatgaagaggattgaagagggtataaaagaactggggtcccaaatccttaaggaacacccagttgaaaacacccagcttcagaatgagaagctctacctgtactacctgcagaacggcagggacatgtacgtggatcaggaactggacatcaatcggctctccgactacgacgtggacgctatcgtgccccagtcttttctcaaagatgattctattgataataaagtgttgacaagatccgataaaaacagagggaagagtgataacgtcccctcagaagaagttgtcaagaaaatgaaaaattattggcggcagctgctgaacgccaaactgatcacacaacggaagttcgataatctgactaaggctgaacgaggtggcctgtctgagttggataaagccggtttcatcaaaaggcagcttgttgagacacgccagatcaccaagcacgtggcccaaattctcgattcacgcatgaacaccaagtacgatgaaaatgacaaactgattcgagaggtgaaagttattactctgaagtctaagctggtctcagatttcagaaaggactttcagttttataaggtgagagagatcaacaattaccaccatgcgcatgatgcctacctgaatgcagtggtaggcactgcacttatcaaaaaatatcccaagcttgaatctgaatttgtttacggagactataaagtgtacgatgttaggaaaatgatcgcaaagtctgagcaggaaataggcaaggccaccgctaagtacttcttttacagcaatattatgaattttttcaagaccgagattacactggccaatggagagattcggaagcgaccacttatcgaaacaaacggagaaacaggagaaatcgtgtgggacaagggtagggatttcgcgacagtccggaaggtcctgtccatgccgcaggtgaacatcgttaaaaagaccgaagtacagaccggaggtttctccaaggaaagtatcctcccgaaaaggaacagcgacaagctgatcgcacgcaaaaaagattgggaccccaagaaatacggcggattcgattctcctacagtcgcttacagtgtactggttgtggccaaagtggagaaagggaagtctaaaaaactcaaaagcgtcaaggaactgctgggcatcacaatcatggagcgatcaagcttcgaaaaaaaccccatcgactttctcgaggcgaaaggatataaagaggtcaaaaaagacctcatcattaagcttcccaagtactctctctttgagcttgaaaacggccggaaacgaatgctcgctagtgcgggcgtgctgcagaaaggtaacgagctggcactgccctctaaatacgttaatttcttgtatctggccagccactatgaaaagctcaaagggtctcccgaagataatgagcagaagcagctgttcgtggaacaacacaaacactaccttgatgagatcatcgagcaaataagcgaattctccaaaagagtgatcctcgccgacgctaacctcgataaggtgctttctgcttacaataagcacagggataagcccatcagggagcaggcagaaaacattatccacttgtttactctgaccaacttgggcgcgcctgcagccttcaagtacttcgacactaccatagacagaaagcggtacacctctacaaaggaggtcctggacgccacactgattcatcagtcaattacggggctctatgaaacaagaatcgacctctctcagctcggtggagacggcggcggcgccggcatggtgcttggcaaaccgcaaacagacccgactctcgaatggttcttgtctcattgccacattcataagtacccatccaagagcacgcttattcaccagggtgaaaaagcggaaacgctgtactacatcgttaaaggctctgtggcagtgctgatcaaagacgaagagggtaaagaaatgatcctctcctatctgaatcagggtgattttattggcgaactgggcctgtttgaagagggccaggaacgtagcgcatgggtacgtgcgaaaaccgcctgtgaagtggctgaaatttcgtacaaaaaatttcgccaattgattcaggtaaacccggacattctgatgcgtttgtctgcacagatggcgcgtcgtctgcaagtcacttcagagaaagtgggcaacctggcgttcctcgacgtgacgggccgcattgcacagactctgctgaatctggcaaaacaaccagacgctatgactcacccggacggtatgcaaatcaaaattacccgtcaggaaattggtcagattgtcggctgttctcaccaccaccaccaccactaaccggcactagctcgagtaaggatctccaggcatcaaataaaacgaaaggctcagtcgaaagactgggcctttcgttttatctgttgtttgtcggtgaacgctctctactagagtcacactggctcaccttcgggtgggcctttctgcgtttatacctagggatatattccgcttcctcggcgaccggttaaagatctttgacagctagctcagtcctaggtataatactagtcatctaattcaacaagaattgttttagagctagaaatagcaagttaaaataaggctagtccgttatcaacttgaaaaagtggcaccgagtcggtgcttttttgcggccgcctcgaggaagcttgggcccgaacaaaaactcatctcagaagaggatctgaatagcgccgtcgaccatcatcatcatcatcattgagtttaaacggtctccagcttggctgttttggcggatgagagaagattttcagcctgatacagattaaatcagaacgcagaagcggtctgataaaacagaatttgcctggcggcagtagcgcggtggtcccacctgaccccatgccgaactcagaagtgaaacgccgtagcgccgatggtagtgtggggtctccccatgcgagagtagggaactgccaggcatcaaataaaacgaaaggctcagtcgaaagactgggcctttcgttttatctgttgtttgtcggtgaact

SEQ ID NO: 36 - DNA, 10023 bp, synthetic construct; identical to SEQ ID NO: 34
  source 1..10023: mol_type = other DNA